European Patent Application EP 4 674 948 A1, published January 7, 2026. Title: AKKERMANSIA MUCINIPHILA AKK11 WITH EFFECT OF REGULATING BLOOD GLUCOSE AND BLOOD LIPID, AND USE THEREOF. Applicant: WECARE PROBIOTICS CO., LTD. The sequence listing filed with the application follows.

SEQUENCE LISTING (1 sequence)

SEQ ID NO: 1 - DNA, 1408 bp, synthetic construct
  source 1..1408: mol_type = other DNA
agtcgaacgagagaattgctagcttgctaataattctctagtggcgcacgggtgagtaacacgtgagtaacctgcccccgagagcgggatagccctgggaaactgggattaataccgcatagtatcgaaagattaaagcagcaatgcgcttggggatgggctcgcggcctattagttagttggtgaggtaacggctcaccaaggcgatgacgggtagccggtctgagaggatgtccggccacactggaactgagacacggtccagacacctacgggtggcagcagtcgagaatcattcacaatgggggaaaccctgatggtgcgacgccgcgtgggggaatgaaggtcttcggattgtaaacccctgtcatgtgggagcaaattaaaaagatagtaccacaagaggaagagacggctaactctgtgccagcagccgcggtaatacagaggtctcaagcgttgttcggaatcactgggcgtaaagcgtgcgtaggctgtttcgtaagtcgtgtgtgaaaggcgcgggctcaacccgcggacggcacatgatactgcgagactagagtaatggagggggaaccggaattctcggtgtagcagtgaaatgcgtagatatcgagaggaacactcgtggcgaaggcgggttcctggacattaactgacgctgaggcacgaaggccaggggagcgaaagggattagatacccctgtagtcctggcagtaaacggtgcacgcttggtgtgcggggaatcgaccccctgcgtgccggagctaacgcgttaagcgtgccgcctggggagtacggtcgcaagattaaaactcaaagaaattgacggggacccgcacaagcggtggagtatgtggcttaattcgatgcaacgcgaagaaccttacctgggcttgacatgtaatgaacaacatgtgaaagcatgcgactcttcggaggcgttacacaggtgctgcatggccgtcgtcagctcgtgtcgtgagatgtttggttaagtccagcaacgagcgcaacccctgttgccagttaccagcacgtgaaggtggggactctggcgagactgcccagatcaactgggaggaaggtggggacgacgtcaggtcagtatggcccttatgcccagggctgcacacgtactacaatgcccagtacagagggggccgaagccgcgaggcggaggaaatcctaaaaactgggcccagttcggactgtaggctgcaacccgcctacacgaagccggaatcgctagtaatggcgcatcagctacggcgccgtgaatacgttcccgggtcttgtacacaccgcccgtcacatcatggaagccggtcgcacccgaagtatctgaagccaaccgcaaggaggcagggtcctaaggtgagactggtaactgggatgaagtcg